European Patent Application EP 4 458 862 A1, published November 6, 2024. Title: BISPECIFIC T-CELL ENGAGER, RECOMBINANT ONCOLYTIC VIRUS THEREOF, AND USE THEREOF. Applicant: SHANGHAI SINOBAY BIOTECHNOLOGY CO., LTD. The sequence listing filed with the application follows.

SEQUENCE LISTING (44 sequences)

SEQ ID NO: 1 - protein, 5 aa, Artificial Sequence
  Heavy chain variable region complementarity determining region 1 (VH CDR1)
GYGMS

SEQ ID NO: 2 - protein, 17 aa, Artificial Sequence
  Heavy chain variable region complementarity determining region 2 (VH CDR2)
TITSGGTYTYYPDSVKG

SEQ ID NO: 3 - protein, 9 aa, Artificial Sequence
  Heavy chain variable region complementarity determining region 3 (VH CDR3)
SLAGNAMDY

SEQ ID NO: 4 - protein, 11 aa, Artificial Sequence
  Light chain variable region complementarity determining region 1 (VL CDR1)
RASQSISSWLA

SEQ ID NO: 5 - protein, 8 aa, Artificial Sequence
  Light chain variable region complementarity determining region 2 (VL CDR2)
KASSLESG

SEQ ID NO: 6 - protein, 5 aa, Artificial Sequence
  Light chain variable region complementarity determining region 3 (VL CDR3)
QHRRA

SEQ ID NO: 7 - protein, 11 aa, Artificial Sequence
  Light chain variable region complementarity determining region 1 (VL CDR1)
RASQGVTSNLA

SEQ ID NO: 8 - protein, 7 aa, Artificial Sequence
  Light chain variable region complementarity determining region 2 (VL CDR2)
GASTRAT

SEQ ID NO: 9 - protein, 5 aa, Artificial Sequence
  Light chain variable region complementarity determining region 3 (VL CDR3)
QHRGT

SEQ ID NO: 10 - protein, 11 aa, Artificial Sequence
  Light chain variable region complementarity determining region 1 (VL CDR1)
RASQGISSRLA

SEQ ID NO: 11 - protein, 7 aa, Artificial Sequence
  Light chain variable region complementarity determining region 2 (VL CDR2)
AASSLQS

SEQ ID NO: 12 - protein, 5 aa, Artificial Sequence
  Light chain variable region complementarity determining region 3 (VL CDR3)
QQANS

SEQ ID NO: 13 - protein, 11 aa, Artificial Sequence
  Light chain variable region complementarity determining region 1 (VL CDR1)
RASQSISNWVA

SEQ ID NO: 14 - protein, 7 aa, Artificial Sequence
  Light chain variable region complementarity determining region 2 (VL CDR2)
KASTLAN

SEQ ID NO: 15 - protein, 5 aa, Artificial Sequence
  Light chain variable region complementarity determining region 3 (VL CDR3)
QHRVT

SEQ ID NO: 16 - protein, 11 aa, Artificial Sequence
  Light chain variable region complementarity determining region 1 (VL CDR1)
RASQSISNWLA

SEQ ID NO: 17 - protein, 7 aa, Artificial Sequence
  Light chain variable region complementarity determining region 2 (VL CDR2)
KASNLES

SEQ ID NO: 18 - protein, 5 aa, Artificial Sequence
  Light chain variable region complementarity determining region 3 (VL CDR3)
QQFGT

SEQ ID NO: 19 - protein, 118 aa, Artificial Sequence
  Heavy chain variable region of CD47 antibody (VHalphaCD47)
EVQLVESGGGLVQPGGSLRLSCAASGFTFSGYGMSWVRQAPGKGLEWVATITSGGTYTYYPDSVKGRFTISRDNAKNSLYLQMNSLRAEDTAVYYCARSLAGNAMDYWGQGTLVTVSS

SEQ ID NO: 20 - protein, 103 aa, Artificial Sequence
  Light chain variable region of CD47 antibody (VLalphaCD47)
DIQMTQSPSTLSASVGDRVTITCRASQSISSWLAWYQQKPGKAPKLLIYKASSLESGVPSRFSGSGSGTEFTLTISSLQPDDFATYYCQHRRAFGQGTKVEIK

SEQ ID NO: 21 - protein, 103 aa, Artificial Sequence
  Light chain variable region of CD47 antibody (VLalphaCD47)
EIVLTQSPVTLSVSPGERATLSCRASQGVTSNLAWYQQKPGQAPRLLIYGASTRATGVPARFSGSGSGTEFTLTISSLQSEDFAVYYCQHRGTFGQGTKVDIK

SEQ ID NO: 22 - protein, 103 aa, Artificial Sequence
  Light chain variable region of CD47 antibody (VLalphaCD47)
DIQMTQSPSSVSASVGDRVTITCRASQGISSRLAWYQQKPGKAPKLLIYAASSLQSGVPSRFSGSGSGTDFTLTISSLQPEDFATYYCQQANSFGGGTKVEIK

SEQ ID NO: 23 - protein, 103 aa, Artificial Sequence
  Light chain variable region of CD47 antibody (VLalphaCD47)
DIQMTQSPTTLSASVGHRVTINCRASQSISNWVAWYQQKAGSAPKLLIYKASTLANGVPSRFSGSGSGTEFILTISSLQPEDVATYYCQHRVTFGPGTKVDLK

SEQ ID NO: 24 - protein, 103 aa, Artificial Sequence
  Light chain variable region of CD47 antibody (VLalphaCD47)
DIQMTQSPSTLSASVGDRVTITCRASQSISNWLAWYQQKPGEAPKLLIYKASNLESGVPSRFSGSGSGTEFTLTISSLQPDDFATYYCQQFGTFGQGTKVEIK

SEQ ID NO: 25 - protein, 119 aa, Artificial Sequence
  Heavy chain variable region of CD3 antibody (VHalphaCD3)
QVQLVQSGAEVKKPGASVKVSCKASGYTFTRYTMHWVRQAPGQGLEWMGYINPSRGYTNYNQKFKDRVTITADKSTSTAYMELSSLRSEDTAVYYCARYYDDHYCLDYWGQGTTVTVSS

SEQ ID NO: 26 - protein, 106 aa, Artificial Sequence
  Light chain variable region of CD3 antibody (VLalphaCD3)
EIVLTQSPATLSLSPGERATLSCSASSSVSYMNWYQQKPGKAPKRLIYDTSKLASGVPSRFSGSGSGTDFTLTINSLEAEDAATYYCQQWSSNPFTFGQGTKVEIK

SEQ ID NO: 27 - protein, 122 aa, Artificial Sequence
  Heavy chain variable region of CD3 antibody (VHalphaCD3)
EVQLVESGGGLVQPKGSLKLSCAASGFTFNTYAMNWVRQAPGKGLEWVARSKYNNYATYYADSVKDRFTISRDDSQSILYLQMNNLKTEDTAMYYCVRHGNFNSYVSWFAYWGQGTLVTVSS

SEQ ID NO: 28 - protein, 110 aa, Artificial Sequence
  Light chain variable region of CD3 antibody (VLalphaCD3)
GSQAVVTQESALTTSPGETVTLTCRSSTGAVTTSNYANWVQEKPDHLFTGLIGGTNKRAPGVPARFSGSLIGKAALTITGAQTEDEAIYFCALWYSNLWVFGGGTKLTVL

SEQ ID NO: 29 - protein, 118 aa, Artificial Sequence; identical to SEQ ID NO: 19
  Heavy chain variable region of B6H12

SEQ ID NO: 30 - protein, 107 aa, Artificial Sequence
  Light chain variable region of B6H12
EIVLTQSPATLSLSPGERATLSCRASQTISDYLHWYQQKPGQAPRLLIKFASQSISGIPARFSGSGSGTDFTLTISSLEPEDFAVYYCQNGHGFPRTFGQGTKVEIK

SEQ ID NO: 31 - DNA, 309 bp, Artificial Sequence
  Light chain variable region of CD47 antibody (VLalphaCD47)
gacattcagatgacacagtctccatctacactgtccgcctccgtgggcgaccgggtgaccattacatgccgcgcctctcagtctattagctcttggctcgcctggtatcagcagaagcccggcaaggcccctaagctgctgatttacaaggcctccagtctggaatctggcgtgccatctaggttcagcggctctggcagcggcaccgagttcacactcacaatttcttccttacagcccgacgacttcgccacatactactgccagcaccggagagccttcggccagggcacaaaggtggagatcaag

SEQ ID NO: 32 - DNA, 309 bp, Artificial Sequence
  Light chain variable region of CD47 antibody (VLalphaCD47)
gagatcgtgctgacccagtctccagtgacactgagcgtgtcccctggcgagagagccaccctgtcttgcagagcctctcagggcgtgacatctaacctcgcctggtatcagcagaagcctggccaggccccaagactcctgatttacggcgcctctacacgcgccacaggcgtgcccgcccggttcagcggctctggctccggcaccgagttcacactcacaattagctctcttcagtccgaggacttcgccgtgtactactgccagcaccgcggcacattcggccagggcacaaaggtggacattaag

SEQ ID NO: 33 - DNA, 309 bp, Artificial Sequence
  Light chain variable region of CD47 antibody (VLalphaCD47)
gacattcagatgacacagtccccatctagcgtgtctgcctccgtgggcgaccgggtgacaattacatgccgcgcctctcagggcattagctcacggctcgcctggtatcagcagaagcctggcaaggcccctaagctgctgatttacgccgcctcttccctccagagcggcgtgccatctaggttctctggctccggctctggcaccgacttcacactgaccatttcttcccttcaacccgaggacttcgccacatactactgccagcaggccaactccttcggcggcggcacaaaggtggagatcaag

SEQ ID NO: 34 - DNA, 309 bp, Artificial Sequence
  Light chain variable region of CD47 antibody (VLalphaCD47)
gacatccagatgacacagtctcctacaacactgagcgcctccgtgggccacagagtgacaattaactgccgcgcctctcagtctatctctaactgggtggcctggtatcagcagaaggccggctccgccccaaagctgctgatttacaaggcctctacactcgccaacggcgtgcctagccggttcagcggctccggctctggcaccgagttcattctcaccatttcttccttgcaacccgaggacgtggccacatactactgccagcacagggtgaccttcggcccaggcaccaaggtggacctcaag

SEQ ID NO: 35 - DNA, 309 bp, Artificial Sequence
  Light chain variable region of CD47 antibody (VLalphaCD47)
gacattcagatgacacagtccccatccaccctgagcgcctccgtgggcgacagagtgaccattacatgccgcgcctctcagtctatttccaactggctcgcctggtatcagcagaagccaggcgaggcccctaagctgctgatttacaaggcctctaacttggagtctggcgtgccatctaggttctccggcagcggctccggcaccgagttcacactcacaattagctctttacaacccgacgacttcgccacatactactgccagcagttcggcaccttcggccagggcacaaaggtggagatcaag

SEQ ID NO: 36 - DNA, 354 bp, Artificial Sequence
  Heavy chain variable region of CD47 antibody (VHalphaCD47)
gaggtgcagctggtggagtctggcggcggcctcgtgcagcctggcggctccctgagactgtcctgcgccgcctctggcttcacattctccggctacggcatgtcttgggtgagacaggccccaggcaagggcctagagtgggtggccacaattacatccggcggcacatacacctactaccccgacagcgtgaagggcagattcaccatttcccgcgacaacgccaagaactctctgtacctccagatgaacagcctgagagccgaggacaccgccgtgtactactgcgcccggtcactcgccggcaacgctatggactactggggccagggcacactcgtgaccgtgtctagc

SEQ ID NO: 37 - DNA, 380 bp, Artificial Sequence
  CMV enhancer or/and other cis-acting elements (E1)
gacattgattattgactagttattaatagtaatcaattacggggtcattagttcatagcccatatatggagttccgcgttacataacttacggtaaatggcccgcctggctgaccgcccaacgacccccgcccattgacgtcaataatgacgtatgttcccatagtaacgccaatagggactttccattgacgtcaatgggtggagtatttacggtaaactgcccacttggcagtacatcaagtgtatcatatgccaagtacgccccctattgacgtcaatgacggtaaatggcccgcctggcattatgcccagtacatgaccttatgggactttcctacttggcagtacatctacgtattagtcatcgctattaccatg

SEQ ID NO: 38 - DNA, 204 bp, Artificial Sequence
  Promoter for recombinant expression (E2)
gtgatgcggttttggcagtacatcaatgggcgtggatagcggtttgactcacggggatttccaagtctccaccccattgacgtcaatgggagtttgttttggcaccaaaatcaacgggactttccaaaatgtcgtaacaactccgccccattgacgcaaatgggcggtaggcgtgtacggtgggaggtctatataagcagagct

SEQ ID NO: 39 - DNA, 331 bp, Artificial Sequence
  5' untranslated region (E3)
cgtttagtgaaccgtcagatcgcctggagacgccatccacgctgttttgacctccatagaagacaccgggaccgatccagcctccgcggccgggaacggtgcattggaacgcggattccccgtgccaagagtgacgtaagtaccgcctatagagtctataggcccacccccttggcttcgttagaacgcggctacaattaatacataaccttatgtatcatacacatacgatttaggtgacactatagaataacatccactttgcctttctctccacaggtgtccactcccaggtccaactgcacctcggttctatcgattgaattccacc

SEQ ID NO: 40 - DNA, 45 bp, Artificial Sequence
  Coding nucleotide sequence of signal peptide of BiTE protein (E4)
atgggatggtcatgtatcatcctttttctagtagcaactgcaacc

SEQ ID NO: 41 - DNA, 20 bp, Artificial Sequence
  3' untranslated region (E6)
aagcttggccgccatggccc

SEQ ID NO: 42 - DNA, 135 bp, Artificial Sequence
  SV40 transcription termination signal region (E7)
aacttgtttattgcagcttataatggttacaaataaagcaatagcatcacaaatttcacaaataaagcatttttttcactgcattctagttgtggtttgtccaaactcatcaatgtatcttatcatgtctggatc

SEQ ID NO: 43 - DNA, 37 bp, Artificial Sequence
  alphaCD47-alphaCD3-BITE-F
gtaccaggcctagtactatggagaggacccttgtctg

SEQ ID NO: 44 - DNA, 36 bp, Artificial Sequence
  alphaCD47-alphaCD3-BITE-R
aataagctcgaagtcgacctaggagagatgctgatg